European Patent Application EP 4 282 880 A1, published November 29, 2023. Title: FULLY HUMAN BROAD-SPECTRUM NEUTRALIZING ANTIBODY 76E1 AGAINST CORONAVIRUS, AND USE THEREOF. Applicant: CENTER FOR EXCELLENCE IN MOLECULAR CELL SCIENCE, CHINESE ACADEMY OF SCIENCES. The sequence listing filed with the application follows.

SEQUENCE LISTING (11 sequences)

SEQ ID NO: 1 - protein, 121 aa, Homo sapiens
EVQLVESGGGVVQPGGSLRLSCEASGFSFKDYGMHWIRQTPGKGLEWISRISGDTRGTSYVDSVKGRFIVSRDNSRNSLFLQMNSLRSEDTALYYCAALVIVAAGDDFDLWGQGTVVTVSS

SEQ ID NO: 2 - protein, 110 aa, Homo sapiens
QSALTQPLSVSGSPGQSVTISCTGSSSDIGSYNFVSWYRQYPGKAPKVMIYEVNKRPSGVPVRFSGSKSGNTASLTVSGLQHEDEADYYCCSYGGRNNLIFGGGTKLTVL

SEQ ID NO: 3 - protein, 8 aa, Homo sapiens
GFSFKDYG

SEQ ID NO: 4 - protein, 8 aa, Homo sapiens
ISGDTRGT

SEQ ID NO: 5 - protein, 14 aa, Homo sapiens
AALVIVAAGDDFDL

SEQ ID NO: 6 - protein, 9 aa, Homo sapiens
SSDIGSYNF

SEQ ID NO: 7 - protein, 10 aa, Homo sapiens
CSYGGRNNLI

SEQ ID NO: 8 - DNA, 363 bp, Homo sapiens
gaggtgcagctggtggagtctgggggaggcgtggtgcagccgggggggtccctgaggctctcctgtgaagcctctggattcagctttaaagactatggcatgcactggatccgtcagactccagggaagggtctggagtggatctctcgtattagtggagacactagaggcacatcctatgtagactctgtgaagggccgattcatcgtctccagagacaacagcagaaactccttgtttttacaaatgaacagtctgagaagtgaagacaccgccttgtattactgtgcagcattagttattgtagctgccggcgatgattttgatctctggggccaagggacagtggtcaccgtttcttca

SEQ ID NO: 9 - DNA, 330 bp, Homo sapiens
cagtctgccctgactcagcctctctcagtgtccgggtctcctggacagtccgtcaccatctcctgcactggatccagcagtgacattgggagttataattttgtctcctggtatcgacaatatccaggcaaagcccccaaagtcatgatctatgaggtcaataagcggccctcgggggtccctgttcgcttctctggctccaagtctggcaacacggcctccctgaccgtctctgggctccaacatgaggatgaggctgactattactgctgctcatatggaggccgcaacaatttgattttcggcggagggaccaagctgaccgtccta

SEQ ID NO: 10 - protein, 25 aa, SARS-CoV-2
PSKPSKRSFIEDLLFNKVTLADAGF

SEQ ID NO: 11 - protein, 15 aa, SARS-CoV-2
PSKPSKRSFIEDLLF